European Patent Specification EP 3 333 186 B9, published October 4, 2023. Title: Combinatorial gamma 9 delta 2 T cell receptor exchange. Applicant: Gadeta B.V. The sequence listing filed with the application follows.

SEQUENCE LISTING (19 sequences)

SEQ ID NO: 1 - protein, 315 aa, Homo sapiens
MVSLLHASTLAVLGALCVYGAGHLEQPQISSTKTLSKTARLECVVSGITISATSVYWYRERPGEVIQFLVSISYDGTVRKESGIPSGKFEVDRIPETSTSTLTIHNVEKQDIATYYCALWEAQQELGKKIKVFGPGTKLIITDKQLDADVSPKPTIFLPSIAETKLQKAGTYLCLLEKFFPDVIKIHWEEKKSNTILGSQEGNTMKTNDTYMKFSWLTVPEKSLDKEHRCIVRHENNKNGVDQEIIFPPIKTDVITMDPKDNCSKDANDTLLLQLTNTSAYYMYLLLLLKSVVYFAIITCCLLRRTAFCCNGEKS

SEQ ID NO: 2 - protein, 292 aa, Homo sapiens
MERISSLIHLSLFWAGVMSAIELVPEHQTVPVSIGVPATLRCSMKGEAIGNYYINWYRKTQGNTMTFIYREKDIYGPGFKDNFQGDIDIAKNLAVLKILAPSERDEGSYYCACDTLGMGGEYTDKLIFGKGTRVTVEPRSQPHTKPSVFVMKNGTNVACLVKEFYPKDIRINLVSSKKITEFDPAIVISPSGKYNAVKLGKYEDSNSVTCSVQHDNKTVHSTDFEVKTDSTDHVKPKETENTKQPSKSCHKPKAIVHTEKVNMMSLTVLGLRMLFAKTVAVNFLLTAKLFFL

SEQ ID NO: 3 - protein, 16 aa, Homo Sapiens
ALWEAQQELGKKIKVF

SEQ ID NO: 4 - protein, 16 aa, Homo Sapiens
ACDTLGMGGEYTDKLI

SEQ ID NO: 5 - DNA, 948 bp, Homo sapiens
atggtgtccctgctgcacgccagcaccctggccgtgctgggcgccctgtgcgtgtatggcgccggacacctggaacagccccagatcagcagcaccaagaccctgagcaagaccgccaggctggaatgcgtggtgtccggcatcaccatcagcgccacctccgtgtactggtacagagagagacccggcgaggtcatccagttcctggtgtccatcagctacgacggcaccgtgcggaaagagagcggcatccccagcggcaagttcgaggtggacagaatccccgagaccagcacctccaccctgaccatccacaacgtggagaagcaggacatcgccacctactactgcgccctgtgggaggcccagcaggaactgggcaagaaaatcaaggtgttcggccctggcaccaagctgatcatcaccgacaagcagctggacgccgacgtgagccccaagcctaccatcttcctgcccagcatcgccgagaccaagctgcagaaggccggcacctacctgtgcctgctggaaaagttcttccccgacgtgatcaagatccactgggaggaaaagaagagcaacaccatcctgggcagccaggaaggcaataccatgaaaaccaacgacacctacatgaagttcagctggctgaccgtgcccgagaagagcctggacaaagagcacagatgcatcgtccggcacgagaacaacaagaacggcgtggaccaggaaatcatcttcccccccatcaagaccgatgtgatcacaatggaccccaaggacaactgcagcaaggacgccaacgataccctgctgctgcagctgaccaacaccagcgcctactacatgtatctcctgctgctgctgaagagcgtggtgtacttcgccatcatcacctgctgtctgctgcggcggaccgccttctgctgcaacggcgagaagagctga

SEQ ID NO: 6 - DNA, 879 bp, Homo sapiens
atggagcggatcagcagcctgatccacctgagcctgttctgggccggagtgatgagcgccatcgagctggtgcccgagcaccagaccgtgcccgtgagcatcggcgtgcccgccaccctgcggtgcagcatgaagggcgaggccatcggcaactactacatcaactggtacagaaagacccagggcaacaccatgaccttcatctaccgggagaaggacatctacggccctggcttcaaggacaacttccagggcgacatcgacatcgccaagaacctggccgtgctgaagatcctggcccccagcgagagggacgagggcagctactactgcgcctgcgacaccctgggcatgggcggcgagtacaccgacaagctgatcttcggcaagggcacccgggtgaccgtggagcccagaagccagccccacaccaagcccagcgtgttcgtgatgaagaacggcaccaacgtggcctgcctggtgaaagagttctaccccaaggacatccggatcaacctggtgtccagcaagaagatcaccgagttcgaccccgccatcgtgatcagccccagcggcaagtacaacgccgtgaagctgggcaagtacgaggacagcaacagcgtgacctgcagcgtgcagcacgacaacaagaccgtgcacagcaccgacttcgaggtgaaaaccgactccaccgaccacgtgaagcccaaagagaccgagaacaccaagcagcccagcaagagctgccacaagcccaaggccatcgtgcacaccgagaaggtgaacatgatgagcctgaccgtgctgggcctgcggatgctgttcgccaagacagtggccgtgaacttcctgctgaccgccaagctgttcttcctgtga

SEQ ID NO: 7 - DNA, 943 bp, Homo sapiens
atggtgtccctgctgcacgccagcaccctggccgtgctgggcgccctgtgcgtgtatggcgccggacacctggaacagccccagatcagcagcaccaagaccctgagcaagaccgccaggctggaatgcgtggtgtccggcatcaccatcagcgccacctccgtgtactggtacagagagagacccggcgaggtcatccagttcctggtgtccatcagctacgacggcaccgtgcggaaagagagcggcatccccagcggcaagttcgaggtggacagaatccccgagaccagcacctccaccctgaccatccacaacgtggagaagcaggacatcgccacctactactgcgccctgtgggaggaggaactgggcaagaaaatcaaggtgttcggccctggcaccaagctgatcatcaccgacaagcagctggacgccgacgtgagccccaagcctaccatcttcctgcccagcatcgccgagaccaagctgcagaaggccggcacctacctgtgcctgctggaaaagttcttccccgacgtgatcaagatccactgggaggaaaagaagagcaacaccatcctgggcagccaggaaggcaataccatgaaaaccaacgacacctacatgaagttcagctggctgaccgtgcccgagaagagcctggacaaagagcacagatgcatcgtccggcacgagaacaacaagaacggcgtggaccaggaaatcatcttcccccccatcaagaccgatgtgatcacaatggaccccaaggacaactgcagcaaggacgccaacgataccctgctgctgcagctgaccaacaccagcgcctactacatgtatctcctgctgctgctgaagagcgtggtgtacttcgccatcatcacctgctgtctgctgcggcggaccgccttctgctgcaacggcgagaagagctgag

SEQ ID NO: 8 - protein, 313 aa, Homo sapiens
MVSLLHASTLAVLGALCVYGAGHLEQPQISSTKTLSKTARLECVVSGITISATSVYWYRERPGEVIQFLVSISYDGTVRKESGIPSGKFEVDRIPETSTSTLTIHNVEKQDIATYYCALWEEELGKKIKVFGPGTKLIITDKQLDADVSPKPTIFLPSIAETKLQKAGTYLCLLEKFFPDVIKIHWEEKKSNTILGSQEGNTMKTNDTYMKFSWLTVPEKSLDKEHRCIVRHENNKNGVDQEIIFPPIKTDVITMDPKDNCSKDANDTLLLQLTNTSAYYMYLLLLLKSVVYFAIITCCLLRRTAFCCNGEKS

SEQ ID NO: 9 - DNA, 867 bp, Homo sapiens
atggagcggatcagcagcctgatccacctgagcctgttctgggccggagtgatgagcgccatcgagctggtgcccgagcaccagaccgtgcccgtgagcatcggcgtgcccgccaccctgcggtgcagcatgaagggcgaggccatcggcaactactacatcaactggtacagaaagacccagggcaacaccatgaccttcatctaccgggagaaggacatctacggccctggcttcaaggacaacttccagggcgacatcgacatcgccaagaacctggccgtgctgaagatcctggcccccagcgagagggacgagggcagctactactgcgcctgcgacctgctgggctacaccgacaagctgatcttcggcaagggcacccgggtgaccgtggagcccagaagccagccccacaccaagcccagcgtgttcgtgatgaagaacggcaccaacgtggcctgcctggtgaaagagttctaccccaaggacatccggatcaacctggtgtccagcaagaagatcaccgagttcgaccccgccatcgtgatcagccccagcggcaagtacaacgccgtgaagctgggcaagtacgaggacagcaacagcgtgacctgcagcgtgcagcacgacaacaagaccgtgcacagcaccgacttcgaggtgaaaaccgactccaccgaccacgtgaagcccaaagagaccgagaacaccaagcagcccagcaagagctgccacaagcccaaggccatcgtgcacaccgagaaggtgaacatgatgagcctgaccgtgctgggcctgcggatgctgttcgccaagacagtggccgtgaacttcctgctgaccgccaagctgttcttcctgtga

SEQ ID NO: 10 - protein, 288 aa, Homo sapiens
MERISSLIHLSLFWAGVMSAIELVPEHQTVPVSIGVPATLRCSMKGEAIGNYYINWYRKTQGNTMTFIYREKDIYGPGFKDNFQGDIDIAKNLAVLKILAPSERDEGSYYCACDLLGYTDKLIFGKGTRVTVEPRSQPHTKPSVFVMKNGTNVACLVKEFYPKDIRINLVSSKKITEFDPAIVISPSGKYNAVKLGKYEDSNSVTCSVQHDNKTVHSTDFEVKTDSTDHVKPKETENTKQPSKSCHKPKAIVHTEKVNMMSLTVLGLRMLFAKTVAVNFLLTAKLFFL

SEQ ID NO: 11 - DNA, 946 bp, Homo sapiens
atggtgtccctgctgcacgccagcaccctggccgtgctgggcgccctgtgcgtgtatggcgccggacacctggaacagccccagatcagcagcaccaagaccctgagcaagaccgccaggctggaatgcgtggtgtccggcatcaccatcagcgccacctccgtgtactggtacagagagagacccggcgaggtcatccagttcctggtgtccatcagctacgacggcaccgtgcggaaagagagcggcatccccagcggcaagttcgaggtggacagaatccccgagaccagcacctccaccctgaccatccacaacgtggagaagcaggacatcgccacctactactgcgccctgtgggagatccaggaactgggcaagaaaatcaaggtgttcggccctggcaccaagctgatcatcaccgacaagcagctggacgccgacgtgagccccaagcctaccatcttcctgcccagcatcgccgagaccaagctgcagaaggccggcacctacctgtgcctgctggaaaagttcttccccgacgtgatcaagatccactgggaggaaaagaagagcaacaccatcctgggcagccaggaaggcaataccatgaaaaccaacgacacctacatgaagttcagctggctgaccgtgcccgagaagagcctggacaaagagcacagatgcatcgtccggcacgagaacaacaagaacggcgtggaccaggaaatcatcttcccccccatcaagaccgatgtgatcacaatggaccccaaggacaactgcagcaaggacgccaacgataccctgctgctgcagctgaccaacaccagcgcctactacatgtatctcctgctgctgctgaagagcgtggtgtacttcgccatcatcacctgctgtctgctgcggcggaccgccttctgctgcaacggcgagaagagctgag

SEQ ID NO: 12 - protein, 314 aa, Homo sapiens
MVSLLHASTLAVLGALCVYGAGHLEQPQISSTKTLSKTARLECVVSGITISATSVYWYRERPGEVIQFLVSISYDGTVRKESGIPSGKFEVDRIPETSTSTLTIHNVEKQDIATYYCALWEIQELGKKIKVFGPGTKLIITDKQLDADVSPKPTIFLPSIAETKLQKAGTYLCLLEKFFPDVIKIHWEEKKSNTILGSQEGNTMKTNDTYMKFSWLTVPEKSLDKEHRCIVRHENNKNGVDQEIIFPPIKTDVITMDPKDNCSKDANDTLLLQLTNTSAYYMYLLLLLKSVVYFAIITCCLLRRTAFCCNGEKS

SEQ ID NO: 13 - DNA, 873 bp, Homo sapiens
atggagcggatcagcagcctgatccacctgagcctgttctgggccggagtgatgagcgccatcgagctggtgcccgagcaccagaccgtgcccgtgagcatcggcgtgcccgccaccctgcggtgcagcatgaagggcgaggccatcggcaactactacatcaactggtacagaaagacccagggcaacaccatgaccttcatctaccgggagaaggacatctacggccctggcttcaaggacaacttccagggcgacatcgacatcgccaagaacctggccgtgctgaagatcctggcccccagcgagagggacgagggcagctactactgcgcctgcgacgccctgaagagaaccgacaccgacaagctgatcttcggcaagggcacccgggtgaccgtggagcccagaagccagccccacaccaagcccagcgtgttcgtgatgaagaacggcaccaacgtggcctgcctggtgaaagagttctaccccaaggacatccggatcaacctggtgtccagcaagaagatcaccgagttcgaccccgccatcgtgatcagccccagcggcaagtacaacgccgtgaagctgggcaagtacgaggacagcaacagcgtgacctgcagcgtgcagcacgacaacaagaccgtgcacagcaccgacttcgaggtgaaaaccgactccaccgaccacgtgaagcccaaagagaccgagaacaccaagcagcccagcaagagctgccacaagcccaaggccatcgtgcacaccgagaaggtgaacatgatgagcctgaccgtgctgggcctgcggatgctgttcgccaagacagtggccgtgaacttcctgctgaccgccaagctgttcttcctgtga

SEQ ID NO: 14 - protein, 290 aa, Homo sapiens
MERISSLIHLSLFWAGVMSAIELVPEHQTVPVSIGVPATLRCSMKGEAIGNYYINWYRKTQGNTMTFIYREKDIYGPGFKDNFQGDIDIAKNLAVLKILAPSERDEGSYYCACDALKRTDTDKLIFGKGTRVTVEPRSQPHTKPSVFVMKNGTNVACLVKEFYPKDIRINLVSSKKITEFDPAIVISPSGKYNAVKLGKYEDSNSVTCSVQHDNKTVHSTDFEVKTDSTDHVKPKETENTKQPSKSCHKPKAIVHTEKVNMMSLTVLGLRMLFAKTVAVNFLLTAKLFFL

SEQ ID NO: 15 - protein, 6 aa, Homo Sapiens
ALKRTD

SEQ ID NO: 16 - protein, 14 aa, Homo Sapiens
ALWEIQELGKKIKV

SEQ ID NO: 17 - protein, 14 aa, Homo Sapiens
ACDALKRTDTDKLI

SEQ ID NO: 18 - protein, 12 aa, Homo Sapiens
ACDLLGYTDKLI

SEQ ID NO: 19 - protein, 8 aa, Homo Sapiens
TLGMGGEY